European Patent Specification EP 4 074 843 B1, published March 11, 2026. Title: METHOD AND KIT FOR DETECTING HUMAN PAPILLOMAVIRUSES. Applicant: Zhejiang Wolwo Bio-Pharmaceutical Co., Ltd. The sequence listing filed with the application follows.

SEQUENCE LISTING (36 sequences)

SEQ ID NO: 1 - DNA, 24 bp, Artificial Sequence
  misc_feature: W=A or T; R=A or G; Y=C or T;
cwggwrcwgayaatagrgaaaatg

SEQ ID NO: 2 - DNA, 22 bp, Artificial Sequence
  misc_feature: Y=C or T; R=A or G; M=A or C; W=A or T;
yrccatatcmccatcctgwata

SEQ ID NO: 3 - DNA, 22 bp, Artificial Sequence
  misc_feature: R=A or G; W=A or T;
gcracaawcttgaggaccarat

SEQ ID NO: 4 - DNA, 25 bp, Artificial Sequence
  misc_feature: Y=C or T; R=A or G;
ygtgtgctagatacrggttcaaatg

SEQ ID NO: 5 - DNA, 25 bp, Artificial Sequence
  misc_feature: B=C, G or T; Y=C or T;
tgcgtgccaggagabgytaatagac

SEQ ID NO: 6 - DNA, 20 bp, Artificial Sequence
  misc_feature: R=A or G; K=G or T;
rkgtcctgggtrctagatac

SEQ ID NO: 7 - DNA, 20 bp, Artificial Sequence
  misc_feature: Y=C or T; K=G or T; R=A or G;
ccygakgtgrttgacctaca

SEQ ID NO: 8 - DNA, 22 bp, Artificial Sequence
  misc_feature: V=A, C or G; H=A, C or T; R=A or G; Y=C or T;
vvhrtyrgccatgtctcttatg

SEQ ID NO: 9 - DNA, 21 bp, Artificial Sequence
  misc_feature: W=A or T; B=C, G or T;
tgcwgagccbtatggcgattg

SEQ ID NO: 10 - DNA, 20 bp, Artificial Sequence
  misc_feature: M=A or C;
acmccaaaattccactcatc

SEQ ID NO: 11 - DNA, 21 bp, Artificial Sequence
tgtggcctaaacgacgtaaac

SEQ ID NO: 12 - DNA, 24 bp, Artificial Sequence
cgcgtgacatagacatccgtactg

SEQ ID NO: 13 - DNA, 24 bp, Artificial Sequence
  misc_feature: M=A or C; R=A or G;
ggagamgttrctagaactgtatga

SEQ ID NO: 14 - DNA, 20 bp, Artificial Sequence
  misc_feature: Y=C or T; D=A, G or T;
ggydctgygtcccacatttc

SEQ ID NO: 15 - DNA, 23 bp, Artificial Sequence
gtgccaggagaaaatactagact

SEQ ID NO: 16 - DNA, 20 bp, Artificial Sequence
  misc_feature: Y=C or T; S=C or G; B=C, G or T;
yscygbaggtactagataca

SEQ ID NO: 17 - DNA, 21 bp, Artificial Sequence
  misc_feature: Y=C or T; B=C, G or T;
ygcctatggbgattctatgtg

SEQ ID NO: 18 - DNA, 23 bp, Artificial Sequence
  misc_feature: H=A, C or T;
ccactagghgtagcaacatatac

SEQ ID NO: 19 - DNA, 22 bp, Artificial Sequence
  misc_feature: M=A or C; Y=C or T;
ggcmcagggycataacaatggt

SEQ ID NO: 20 - DNA, 20 bp, Artificial Sequence
  misc_feature: D=A, G or T; W=A or T; R=A or G;
dcgwccaagrggatattgat

SEQ ID NO: 21 - DNA, 25 bp, Artificial Sequence
  misc_feature: W=A or T; R=A or G;
gcwgatgtrtatggrgacagtatgt

SEQ ID NO: 22 - DNA, 24 bp, Artificial Sequence
  misc_feature: R=A or G; Y=C or T;
rggcttrttaaayaactgggartc

SEQ ID NO: 23 - DNA, 21 bp, Artificial Sequence
tgtccaccaatgcttattaca

SEQ ID NO: 24 - DNA, 24 bp, Artificial Sequence
  misc_feature: S=C or G; K=G or T;
cctcttcctsgtkcaaatctaatc

SEQ ID NO: 25 - DNA, 22 bp, Artificial Sequence
  misc_feature: W=A or T; Y=C or T;
gatggwaacccaactagyatag

SEQ ID NO: 26 - DNA, 22 bp, Artificial Sequence
ccgttgctgtcaaatggaaatg

SEQ ID NO: 27 - DNA, 25 bp, Artificial Sequence
  misc_feature: S=C or G; Y=C or T;
asygaagtatcctctgttgcgtcta

SEQ ID NO: 28 - DNA, 21 bp, Artificial Sequence
tcgaatcgcactcgctttcta

SEQ ID NO: 29 - DNA, 22 bp, Artificial Sequence
  misc_feature: W=A or T; K=G or T;
gttgtwagcackgatgaatatg

SEQ ID NO: 30 - DNA, 22 bp, Artificial Sequence
  misc_feature: R=A or G; Y=C or T;
ccactaatrccyacaccyaatg

SEQ ID NO: 31 - DNA, 22 bp, Artificial Sequence
  misc_feature: R=A or G;
gacgtgarcaratgtttgttag

SEQ ID NO: 32 - DNA, 20 bp, Artificial Sequence
  misc_feature: W=A or T; K=G or T; R=A or G;
ggwggkgtwarrccaaattg

SEQ ID NO: 33 - DNA, 20 bp, Artificial Sequence
  misc_feature: R=A or G; Y=C or T;
trcacgyaracgccgtaaac

SEQ ID NO: 34 - DNA, 20 bp, Artificial Sequence
  misc_feature: K=G or T; Y=C or T; W=A or T;
kkccyacwgcaagtagtcta

SEQ ID NO: 35 - DNA, 22 bp, Artificial Sequence
  misc_feature: M=A or C; W=A or T; R=A or G;
ggcmwtrttagatgatgcwaca

SEQ ID NO: 36 - DNA, 21 bp, Artificial Sequence
cacgttcatacagttctagga